European Patent Application EP 4 501 930 A1, published February 5, 2025. Title: Aromatic ring compound and use thereof. Applicant: SHANGHAI SHIJIANG BIOTECHNOLOGY CO., LTD. Application EP. The sequence listing filed with the application follows.

SEQUENCE LISTING (2 sequences)

SEQ ID NO: 1 - DNA, 2500 bp, synthetic construct
  source 1..2500: mol_type = other DNA
tatccaagagctatcagcactcccatgtttattgtagcactgttcacaatagccaagatttggaagtactctaagtgtccattagcagatgaatggataaagacaatgtggtaatacacataatggagtactattcagtcataaagaagaattagatcctgtcatttgcaataacatggatggaactggaggtcataatgttgagtgaaataaaccaggcacagaaagacaaactttgcatgttctcacttatttatgggagctaaaaactaaaataactgaactcacagagatagagagtagaaggatggttacgagaggatgggaagggtagcgaggtgggtaggggggatgtggggatcattaatgggtataaaaaatagttagaggccaggcgcagtggctcacgcctgtaatcccagcactttgggaggccgaggtaggcggaacacctgaggagttcaagaccagcctggccaatatgatgaaaccccgtctctactaaaaatacaaaaattagctgggcgtgatggtgtgcacctgtagtcccagctgcttgggaggctgaggcaggagaatcgctggaacccaagaggtgaaggttgcagtgagctgagatcgcgtcactgcactccagcctgggtgacagagtgagactccacatcaaaaaaaaaaaaaaaaagttagaaagattgaataagacctaatatttgctagcacaacagggtgaatatagtaaaaaataatttatttgtaccttcaaaaataactagacaagtataattgggttgtttgtaacacacaaaaaataagtacttgaagtggtggataccccatttaccctgatgtgattattttgtattgcaggcctctatcagaatatctcatgtaacccataaatatatacacctactctgtacccacaaaaagtttttaaaaagaaaaataaatagcaaccgaaaaaaaaagagagggagaaaagaaaaaagaaaaaaaaatcaagtgcctggctgggtagaataaattctaaggccacaatgttactgaccatgggttttttggctctcagtgtatagaaattgacacaaggccaatagtcttcccaaacatgctttactggaacttacgccctggcataagggccacaacaaaagagagagcgaattctctggcttgctgactccttggaaaaaaccggtagggatttttttattaggcaaagcacaggaattgacgtcagaggcaggatgtgctgctgggcaaagcatacgagaagtggggtatgcaggtcagcattacttggttgcaatggttatcttgaggaatgggccaactggtggtctggccagtggcaacaaggctgtaaatcaattattcagcattccttcccaaggtgggacacccggcaacattgtttatctcctaaggccagttcctggaattaagtgaaaggatgactaatggacatgttgtcagtgaggtagtggtgtgggttttgtgaccagtgggaatgcacgaaagaatgctttagcggggagtgagctgaagccaagccccatccctactctgtctcaaagtgagttcagaaaaggggatttaaagaattctttttttttttttttttttttttgagacagagtcttgctctgtcgcccaggctggagtgcagtggcgccatcttggctcactgcaagctccgccccccgggttcatgccattctcctgcctcagcctcccaagtagctgggactgcaggtgcctaccaccaagcccagctaattttttgtattttttttttagtagagacggggtttcaccatgttagccaggatggtctcgatctcctgacctcgtgatctgcccgccttagcctcccaaagtgctgggattacaggcatgagcctccgcccccggccttaaataattcttaaaggaagtaaagttaactttgaaagaactatcaggatttggattgactgaaaggagtggggaagcttagggaggaggtgcttgccagacactgggtcatggcagtggtcggtgaagctgcagttgcctagggcagggatggagagagagtctgggcatgaggagagggtctcgggatgtttggctggactagattttacagaaagccttatccaggcttttaaaattactctttccagacttcatctgagactccttcttcagccaacattccttagccctgaatacatttcctatcctcatctttcccttcttttttttcctttcttttacatgtttaaatttaaaccattcttcgtgaccccttttcttgggagattcatggcaagaacgagaagaatgatggtgcttgttaggggatgtcctgtctctctgaactttggggtcctatgcattaaataattttcctgacgagctcaagtgctccctctggtctacaatccctggcggctggccttcatcccttgggcaagcattgcatacagctcatggccctccctctaccataccc

SEQ ID NO: 2 - DNA, 21 bp, synthetic construct
  source 1..21: mol_type = other DNA
gttcttcatctgcaccataaa